European Patent Application EP 4 242 234 A1, published September 13, 2023. Title: ANTI-LAG-3 MONOCLONAL ANTIBODY AND ANTIGEN BINDING FRAGMENT THEREOF, AND USE THEREOF. Applicant: BEIJING DONGFANG BIOTECH CO., LTD. BEIJING JINGYITAIXIANG TECHNOLOGY DEVELOPMENAT CO., LTD. The sequence listing filed with the application follows.

SEQUENCE LISTING (47 sequences)

SEQ ID NO: 1 - protein, 5 aa, Artificial Sequence
  Synthesized
DTYMH

SEQ ID NO: 2 - protein, 17 aa, Artificial Sequence
  Synthesized
KIDPANGNTKYDPKFQG

SEQ ID NO: 3 - protein, 8 aa, Artificial Sequence
  Synthesized
DTTVGLDY

SEQ ID NO: 4 - protein, 10 aa, Artificial Sequence
  Synthesized
RASSSVNYMY

SEQ ID NO: 5 - protein, 7 aa, Artificial Sequence
  Synthesized
YTSKLAS

SEQ ID NO: 6 - protein, 9 aa, Artificial Sequence
  Synthesized
QQWSSNPHT

SEQ ID NO: 7 - protein, 7 aa, Artificial Sequence
  Synthesized
YTSNLAP

SEQ ID NO: 8 - protein, 10 aa, Artificial Sequence
  Synthesized
QQFTSSPSMT

SEQ ID NO: 9 - protein, 7 aa, Artificial Sequence
  Synthesized
GYSFTSY

SEQ ID NO: 10 - protein, 17 aa, Artificial Sequence
  Synthesized
WIFPGTGNTRYNEKFKG

SEQ ID NO: 11 - protein, 12 aa, Artificial Sequence
  Synthesized
IGGRLTGDAMDY

SEQ ID NO: 12 - protein, 15 aa, Artificial Sequence
  Synthesized
RASESVDSYGNSFMH

SEQ ID NO: 13 - protein, 7 aa, Artificial Sequence
  Synthesized
LASNLES

SEQ ID NO: 14 - protein, 9 aa, Artificial Sequence
  Synthesized
QQNNEDPWT

SEQ ID NO: 15 - protein, 5 aa, Artificial Sequence
  Synthesized
TYAVH

SEQ ID NO: 16 - protein, 17 aa, Artificial Sequence
  Synthesized
VIWSGGSTDYNTAFISR

SEQ ID NO: 17 - protein, 8 aa, Artificial Sequence
  Synthesized
LDGTFFDY

SEQ ID NO: 18 - protein, 12 aa, Artificial Sequence
  Synthesized
TASSSVSSSYLH

SEQ ID NO: 19 - protein, 7 aa, Artificial Sequence
  Synthesized
STSNLAS

SEQ ID NO: 20 - protein, 9 aa, Artificial Sequence
  Synthesized
HQYHRSPPT

SEQ ID NO: 21 - protein, 117 aa, Artificial Sequence
  Synthesized
EVQLQQSGAELVKPGASVKLSCTASGFNIKDTYMHWVKQRPEQGLEWIGKIDPANGNTKYDPKFQGKATITADTSSNTAYLQLSRLTSEDTAVYYCARDTTVGLDYWGQGTTLTVSS

SEQ ID NO: 22 - protein, 106 aa, Artificial Sequence
  Synthesized
DIVITQSTAIMSASLGEKVTMSCRASSSVNYMYWYQQKSDASPKLWIYYTSKLASGVPARFSGSGSGTSYSLTISSMEAEDAATYYCQQWSSNPHTFGGGTKLEIK

SEQ ID NO: 23 - protein, 107 aa, Artificial Sequence
  Synthesized
DIVLTQTPAIMSASLGEKVTMSCRASSSVNYMYWYQQKSDASPKLWIYYTSNLAPGVPARFSGSGSGNSYSLTISSMEGEDAATYYCQQFTSSPSMTFGGGTKLEIK

SEQ ID NO: 24 - protein, 121 aa, Artificial Sequence
  Synthesized
EVKLEESGPELVKPGASVKISCKASGYSFTSYYIHWVKQRPGQGLEWIGWIFPGTGNTRYNEKFKGKATLTADTSSSTVYMQLSGLTSEDSAVYFCARIGGRLTGDAMDYWGQGTSVTVSS

SEQ ID NO: 25 - protein, 111 aa, Artificial Sequence
  Synthesized
DIVLTQSTASLAVSLGQRATISCRASESVDSYGNSFMHWYQQKPGQPPKLLIYLASNLESGVPARFSGSGSRTDFTLTIDPVEADDAATYYCQQNNEDPWTFGGGTKLEIK

SEQ ID NO: 26 - protein, 116 aa, Artificial Sequence
  Synthesized
QVKLEESGPGLVQPSQSLSITCTVSAFSLTTYAVHWVRQSPGKGLEWLGVIWSGGSTDYNTAFISRLNITKDNSKSQVFFKMNSLQANDTAIYYCARLDGTFFDYWGQGTTLTVSS

SEQ ID NO: 27 - protein, 108 aa, Artificial Sequence
  Synthesized
DIVLTQTPAIMSASLGERVTMTCTASSSVSSSYLHWYQQKPGSSPKLWIYSTSNLASGVPARFSGSGSGTSYSLTISSMEAEDAATYYCHQYHRSPPTFGGGTKLEIK

SEQ ID NO: 28 - protein, 106 aa, Artificial Sequence
  Synthesized
ADAAPTVSIFPPSSEQLTSGGASVVCFLNNFYPKDINVKWKIDGSERQNGVLNSWTDQDSKDSTYSMSSTLTLTKDEYERHNSYTCEATHKTSTSPIVKSFNRNEC

SEQ ID NO: 29 - protein, 323 aa, Artificial Sequence
  Synthesized
AKTTPPSVYPLAPGSAAQTNSMVTLGCLVKGYFPEPVTVTWNSGSLSSGVHTFPAVLQSDLYTLSSSVTVPSSTWPSETVTCNVAHPASSTKVDKKIVPRDCGCKPCICTVPEVSSVFIFPPKPKDVLTITLTPKVTCVVVDISKDDPEVQFSWFVDDVEVHTAQTQPREEQFNSTFRSVSELPIMHQDWLNGKEFKCRVNSAAFPAPIEKTISKTKGRPKAPQVYTIPPPKEQMAKDKVSLTCMITDFFPEDITVEWQWNGQPAENYKNTQPIMDTDGSYFVYSKLNVQKSNWEAGNTFTCSVLHEGLHNHHTEKSLSHSPG

SEQ ID NO: 30 - protein, 330 aa, Artificial Sequence
  Synthesized
AKTTAPSVYPLAPVCGDTTGSSVTLGCLVKGYFPEPVTLTWNSGSLSSGVHTFPAVLQSDLYTLSSSVTVTSSTWPSQSITCNVAHPASSTKVDKKIEPRGPTIKPCPPCKCPAPNLLGGPSVFIFPPKIKDVLMISLSPIVTCVVVDVSEDDPDVQISWFVNNVEVHTAQTQTHREDYNSTLRVVSALPIQHQDWMSGKEFKCKVNNKDLPAPIERTISKPKGSVRAPQVYVLPPPEEEMTKKQVTLTCMVTDFMPEDIYVEWTNNGKTELNYKNTEPVLDSDGSYFMYSKLRVEKKNWVERNSYSCSVVHEGLHNHHTTKSFSRTPGK

SEQ ID NO: 31 - protein, 336 aa, Artificial Sequence
  Synthesized
AKTTPPSVYPLAPGCGDTTGSSVTLGCLVKGYFPESVTVTWNSGSLSSSVHTFPALLQSGLYTMSSSVTVPSSTWPSQTVTCSVAHPASSTTVDKKLEPSGPISTINPCPPCKECHKCPAPNLEGGPSVFIFPPNIKDVLMISLTPKVTCVVVDVSEDDPDVQISWFVNNVEVHTAQTQTHREDYNSTIRVVSTLPIQHQDWMSGKEFKCKVNNKDLPSPIERTISKIKGLVRAPQVYILPPPAEQLSRKDVSLTCLVVGFNPGDISVEWTSNGHTEENYKDTAPVLDSDGSYFIYSKLNMKTSKWEKTDSFSCNVRHEGLKNYYLKKTISRSPGK

SEQ ID NO: 32 - protein, 399 aa, Artificial Sequence
  Synthesized
ATTTAPSVYPLVPGCSDTSGSSVTLGCLVKGYFPEPVTVKWNYGALSSGVRTVSSVLQSGFYSLSSLVTVPSSTWPSQTVICNVAHPASKTELIKRIEPRIPKPSTPPGSSCPPGNILGGPSVFIFPPKPKDALMISLTPKVTCVVVDVSEDDPDVHVSWFVDNKEVHTAWTQPREAQYNSTFRVVSALPIQHQDWMRGKEFKCKVNNKALPAPIERTISKPKGRAQTPQVYTIPPPREQMSKKKVSLTCLVTNFFSEAISVEWERNGELEQDYKNTPPILDSDGTYFLYSKLTVDTDSWLQGEIFTCSVVHEALHNHHTQKNLSRSPELELNETCAEAQDGELDGLWTTITIFISLFLLSVCYSASVTLFKVKWIFSSVVQVKQTAIPDYRNMIGQGA

SEQ ID NO: 33 - protein, 117 aa, Artificial Sequence
  Synthesized
QVQLVQSGAEVKKPGASVKVSCKASGYTFTDTYMHWVRQAPGQGLEWIGKIDPANGNTKYDPKFQGRATITADTSISTAYMELSRLRSDDTAVYYCARDTTVGLDYWGQGTLVTVSS

SEQ ID NO: 34 - protein, 106 aa, Artificial Sequence
  Synthesized
DIVITQSPAFLSVTPGEKVTITCRASSSVNYMYWYQQKPDASPKLWIYYTSKLASGVPSRFSGSGSGTDYTFTISSLEAEDAATYYCQQWSSNPHTFGGGTKVEIK

SEQ ID NO: 35 - protein, 106 aa, Artificial Sequence
  Synthesized
DIVITQSPAFLSVTPGEKVTITCRASSSVNYMYWYQQKPDQAPKLLIYYTSKLASGVPSRFSGSGSGTDYTFTISSLEAEDAATYYCQQWSSNPHTFGGGTKVEIK

SEQ ID NO: 36 - protein, 117 aa, Artificial Sequence
  Synthesized
QVQLVQSGAEVKKPGASVKVSCKASGYNITDTYMHWVRQAPGQGLEWIGKIDPANGNTKYDPKFQGRATITADTSISTAYMELSRLRSDDTAVYYCARDTTVGLDYWGQGTLVTVSS

SEQ ID NO: 37 - protein, 117 aa, Artificial Sequence
  Synthesized
QVQLVQSGAEVKKPGASVKVSCKASGYNIKDTYMHWVKQAPGQGLEWIGKIDPANGNTKYDPKFQGKATITADTSISTAYMELSRLRSDDTAVYYCARDTTVGLDYWGQGTLVTVSS

SEQ ID NO: 38 - protein, 106 aa, Artificial Sequence
  Synthesized
DIVITQSPAFLSVTPGEKVTITCRASSSVNYMYWYQQKPDASPKLWIYYTSKLASGVPARFSGSGSGTSYTFTISSLEAEDAATYYCQQWSSNPHTFGGGTKVEIK

SEQ ID NO: 39 - protein, 330 aa, Artificial Sequence
  Synthesized
ASTKGPSVFPLAPSSKSTSGGTAALGCLVKDYFPEPVTVSWNSGALTSGVHTFPAVLQSSGLYSLSSVVTVPSSSLGTQTYICNVNHKPSNTKVDKRVEPKSCDKTHTCPPCPAPELLGGPSVFLFPPKPKDTLMISRTPEVTCVVVDVSHEDPEVKFNWYVDGVEVHNAKTKPREEQYNSTYRVVSVLTVLHQDWLNGKEYKCKVSNKALPAPIEKTISKAKGQPREPQVYTLPPSREEMTKNQVSLTCLVKGFYPSDIAVEWESNGQPENNYKTTPPVLDSDGSFFLYSKLTVDKSRWQQGNVFSCSVMHEALHNHYTQKSLSLSPGK

SEQ ID NO: 40 - protein, 326 aa, Artificial Sequence
  Synthesized
ASTKGPSVFPLAPCSRSTSESTAALGCLVKDYFPEPVTVSWNSGALTSGVHTFPAVLQSSGLYSLSSVVTVPSSNFGTQTYTCNVDHKPSNTKVDKTVERKCCVECPPCPAPPVAGPSVFLFPPKPKDTLMISRTPEVTCVVVDVSHEDPEVQFNWYVDGVEVHNAKTKPREEQFNSTFRVVSVLTVVHQDWLNGKEYKCKVSNKGLPAPIEKTISKTKGQPREPQVYTLPPSREEMTKNQVSLTCLVKGFYPSDIAVEWESNGQPENNYKTTPPMLDSDGSFFLYSKLTVDKSRWQQGNVFSCSVMHEALHNHYTQKSLSLSPGK

SEQ ID NO: 41 - protein, 327 aa, Artificial Sequence
  Synthesized
ASTKGPSVFPLAPCSRSTSESTAALGCLVKDYFPEPVTVSWNSGALTSGVHTFPAVLQSSGLYSLSSVVTVPSSSLGTKTYTCNVDHKPSNTKVDKRVESKYGPPCPPCPAPEFLGGPSVFLFPPKPKDTLMISRTPEVTCVVVDVSQEDPEVQFNWYVDGVEVHNAKTKPREEQFNSTYRVVSVLTVLHQDWLNGKEYKCKVSNKGLPSSIEKTISKAKGQPREPQVYTLPPSQEEMTKNQVSLTCLVKGFYPSDIAVEWESNGQPENNYKTTPPVLDSDGSFFLYSRLTVDKSRWQEGNVFSCSVMHEALHNHYTQKSLSLSLGK

SEQ ID NO: 42 - protein, 107 aa, Artificial Sequence [sequence omitted]

SEQ ID NO: 43 - protein, 113 aa, Artificial Sequence
  Synthesized
QVQLVESGGGVVQPGRSLRLDCKASGITFSNYGMHWVRQAPGKGLEWVAVIWYDSSRKYYADSVKGRFTISRDNSKNTLFLQMNSLRAEDTAVYYCATNNDYWGQGTLVTVSS

SEQ ID NO: 44 - protein, 107 aa, Artificial Sequence
  Synthesized
DIQMTQSPSSLSASVGDRVTITCRASQSIHNYLDWYQQKPGKAPKLLIYNASTRATGVPSRFSGSGSGTDFTLTISSLQPEDFATYYCQQELHLPLTFGQGTKVEIK

SEQ ID NO: 45 - protein, 107 aa, Artificial Sequence
  Synthesized
DIQMTQSPSSLSASVGDRVTITCRASQSVSNYLDWYQQKPGKAPKLLIYDASTRATGVPSRFSGSGSGTDFTLTISSLQPEDFATYYCQQNMQLPLTFGQGTKVEIK

SEQ ID NO: 46 - protein, 113 aa, Artificial Sequence
  Synthesized
QVQLVESGGGVVQPGRSLRLDCKASGITFSNNGMHWVRQAPGKGLEWVAVIWYDSSRKYYADSVKGRFTISRDNSKNTLFLQMNSLRAEDTAVYYCATNNDYWGQGTLVTVSS

SEQ ID NO: 47 - protein, 113 aa, Artificial Sequence
  Synthesized
QVQLVESGGGVVQPGRSLRLDCKASGITFSNYGMHWVRQAPGKGLEWVAVIWYDGSKKYYADSVKGRFTISRDNSKNTLFLQMNSLRAEDTAVYYCATNNDYWGQGTLVTVSS